European Patent Application EP 4 357 779 A1, published April 24, 2024. Title: INFLAMMATORY DISORDER IN A FELIDAE. Applicant: MARS, INCORPORATED. The sequence listing filed with the application follows.

SEQUENCE LISTING (2 sequences)

SEQ ID NO: 1 - DNA, 15 bp, synthetic construct
  source 1..15: mol_type = other DNA
tacgggaggcagcag

SEQ ID NO: 2 - DNA, 16 bp, synthetic construct
  source 1..16: mol_type = other DNA
ccagggtatctaatcc